European Patent Application EP 4 471 054 A2, published December 4, 2024. Title: 载脂蛋白E的C端片段及其在抑制γ分泌酶酶活中的应用. Applicant: Shanghai Institute of Organic Chemistry, Chinese Academy of Sciences. Application CN. The sequence listing filed with the application follows.

SEQUENCE LISTING (100 sequences)

SEQ ID NO: 1 - DNA, 21 bp, synthetic construct
  source 1..21: mol_type = other DNA
agagcaacatctggggacaaa

SEQ ID NO: 2 - DNA, 22 bp, synthetic construct
  source 1..22: mol_type = other DNA
tccacaaataggttggccagat

SEQ ID NO: 3 - DNA, 20 bp, synthetic construct
  source 1..20: mol_type = other DNA
gctctgggagagccaacata

SEQ ID NO: 4 - DNA, 21 bp, synthetic construct
  source 1..21: mol_type = other DNA
aacgaattggctttgctgtca

SEQ ID NO: 5 - DNA, 21 bp, synthetic construct
  source 1..21: mol_type = other DNA
aggctatggtcatgagggttg

SEQ ID NO: 6 - DNA, 20 bp, synthetic construct
  source 1..20: mol_type = other DNA
tgactctctgcatggtggtg

SEQ ID NO: 7 - DNA, 20 bp, synthetic construct
  source 1..20: mol_type = other DNA
tcagaattgagtgcagggct

SEQ ID NO: 8 - DNA, 20 bp, synthetic construct
  source 1..20: mol_type = other DNA
tttgagcctcccttgactgg

SEQ ID NO: 9 - DNA, 19 bp, synthetic construct
  source 1..19: mol_type = other DNA
ggtattccagtccccgctg

SEQ ID NO: 10 - RNA, 21 nt, synthetic construct
  source 1..21: mol_type = other RNA
gattatctaatggacgacccc

SEQ ID NO: 11 - RNA, 21 nt, synthetic construct
  source 1..21: mol_type = other RNA
gcgtgcttcgctccgtatttg

SEQ ID NO: 12 - protein, 299 aa, synthetic construct
KVEQAVETEPEPELRQQTEWQSGQRWELALGRFWDYLRWVQTLSEQVQEELLSSQVTQELRALMDETMKELKAYKSELEEQLTPVAEETRARLSKELQAAQARLGADMEDVCGRLVQYRGEVQAMLGQSTEELRVRLASHLRKLRKRLLRDADDLQKCLAVYQAGAREGAERGLSAIRERLGPLVEQGRVRAATVGSLAGQPLQERAQAWGERLRARMEEMGSRTRDRLDEVKEQVAEVRAKLEEQAQQIRLQAEAFQARLKSWFEPLVEDMQRQWAGLVEKVQAAVGTSAAPVPSDNH

SEQ ID NO: 13 - protein, 85 aa, synthetic construct
RARMEEMGSRTRDRLDEVKEQVAEVRAKLEEQAQQIRLQAEAFQARLKSWFEPLVEDMQRQWAGLVEKVQAAVGTSAAPVPSDNH

SEQ ID NO: 14 - protein, 86 aa, synthetic construct
LRARMEEMGSRTRDRLDEVKEQVAEVRAKLEEQAQQIRLQAEAFQARLKSWFEPLVEDMQRQWAGLVEKVQAAVGTSAAPVPSDNH

SEQ ID NO: 15 - protein, 87 aa, synthetic construct
RLRARMEEMGSRTRDRLDEVKEQVAEVRAKLEEQAQQIRLQAEAFQARLKSWFEPLVEDMQRQWAGLVEKVQAAVGTSAAPVPSDNH

SEQ ID NO: 16 - protein, 88 aa, synthetic construct
ERLRARMEEMGSRTRDRLDEVKEQVAEVRAKLEEQAQQIRLQAEAFQARLKSWFEPLVEDMQRQWAGLVEKVQAAVGTSAAPVPSDNH

SEQ ID NO: 17 - protein, 89 aa, synthetic construct
GERLRARMEEMGSRTRDRLDEVKEQVAEVRAKLEEQAQQIRLQAEAFQARLKSWFEPLVEDMQRQWAGLVEKVQAAVGTSAAPVPSDNH

SEQ ID NO: 18 - protein, 83 aa, synthetic construct
RMEEMGSRTRDRLDEVKEQVAEVRAKLEEQAQQIRLQAEAFQARLKSWFEPLVEDMQRQWAGLVEKVQAAVGTSAAPVPSDNH

SEQ ID NO: 19 - protein, 82 aa, synthetic construct
MEEMGSRTRDRLDEVKEQVAEVRAKLEEQAQQIRLQAEAFQARLKSWFEPLVEDMQRQWAGLVEKVQAAVGTSAAPVPSDNH

SEQ ID NO: 20 - protein, 81 aa, synthetic construct
EEMGSRTRDRLDEVKEQVAEVRAKLEEQAQQIRLQAEAFQARLKSWFEPLVEDMQRQWAGLVEKVQAAVGTSAAPVPSDNH

SEQ ID NO: 21 - protein, 80 aa, synthetic construct
EMGSRTRDRLDEVKEQVAEVRAKLEEQAQQIRLQAEAFQARLKSWFEPLVEDMQRQWAGLVEKVQAAVGTSAAPVPSDNH

SEQ ID NO: 22 - protein, 79 aa, synthetic construct [sequence omitted]

SEQ ID NO: 23 - protein, 79 aa, synthetic construct
ARMEEMGSRTRDRLDEVKEQVAEVRAKLEEQAQQIRLQAEAFQARLKSWFEPLVEDMQRQWAGLVEKVQAAVGTSAAPV

SEQ ID NO: 24 - protein, 74 aa, synthetic construct
ARMEEMGSRTRDRLDEVKEQVAEVRAKLEEQAQQIRLQAEAFQARLKSWFEPLVEDMQRQWAGLVEKVQAAVGT

SEQ ID NO: 25 - protein, 71 aa, synthetic construct
EEMGSRTRDRLDEVKEQVAEVRAKLEEQAQQIRLQAEAFQARLKSWFEPLVEDMQRQWAGLVEKVQAAVGT

SEQ ID NO: 26 - protein, 70 aa, synthetic construct
EEMGSRTRDRLDEVKEQVAEVRAKLEEQAQQIRLQAEAFQARLKSWFEPLVEDMQRQWAGLVEKVQAAVG

SEQ ID NO: 27 - protein, 69 aa, synthetic construct
EEMGSRTRDRLDEVKEQVAEVRAKLEEQAQQIRLQAEAFQARLKSWFEPLVEDMQRQWAGLVEKVQAAV

SEQ ID NO: 28 - protein, 68 aa, synthetic construct
EEMGSRTRDRLDEVKEQVAEVRAKLEEQAQQIRLQAEAFQARLKSWFEPLVEDMQRQWAGLVEKVQAA

SEQ ID NO: 29 - protein, 67 aa, synthetic construct
EEMGSRTRDRLDEVKEQVAEVRAKLEEQAQQIRLQAEAFQARLKSWFEPLVEDMQRQWAGLVEKVQA

SEQ ID NO: 30 - protein, 66 aa, synthetic construct
EEMGSRTRDRLDEVKEQVAEVRAKLEEQAQQIRLQAEAFQARLKSWFEPLVEDMQRQWAGLVEKVQ

SEQ ID NO: 31 - protein, 61 aa, synthetic construct
EEMGSRTRDRLDEVKEQVAEVRAKLEEQAQQIRLQAEAFQARLKSWFEPLVEDMQRQWAGL

SEQ ID NO: 32 - protein, 56 aa, synthetic construct
EEMGSRTRDRLDEVKEQVAEVRAKLEEQAQQIRLQAEAFQARLKSWFEPLVEDMQR

SEQ ID NO: 33 - protein, 84 aa, synthetic construct
ARMEEMGSRTRDRLDEVKEQVAEVRAKLEEQAQQIRLQAEAFQARLKSWFEPLVEDMQRQWAGLVEKVQAAVGTSAAPVPSDNH

SEQ ID NO: 34 - protein, 60 aa, synthetic construct
EMGSRTRDRLDEVKEQVAEVRAKLEEQAQQIRLQAEAFQARLKSWFEPLVEDMQRQWAGL

SEQ ID NO: 35 - protein, 16 aa, synthetic construct
RQIKIWFQNRRMKWKK

SEQ ID NO: 36 - protein, 11 aa, synthetic construct
YGRKKRRQRRR

SEQ ID NO: 37 - protein, 8 aa, synthetic construct
KQAIPVAK

SEQ ID NO: 38 - protein, 15 aa, synthetic construct
RRRRNRTRRNRRRVR

SEQ ID NO: 39 - protein, 21 aa, synthetic construct
KLTRAQRRAAARKNKRNTRGC

SEQ ID NO: 40 - protein, 21 aa, synthetic construct
ALWKTLLKKVLKAPKKKRKVC

SEQ ID NO: 41 - protein, 9 aa, synthetic construct
RKKRRQRRR

SEQ ID NO: 42 - protein, 34 aa, synthetic construct
DAATATRGRSAASRPTERPRAPARSASRPRRPVE

SEQ ID NO: 43 - protein, 27 aa, synthetic construct
GWTLNSAGYLLGKINLKALAALAKKIL

SEQ ID NO: 44 - protein, 21 aa, synthetic construct
AGYLLGKINLKALAALAKKIL

SEQ ID NO: 45 - protein, 16 aa, synthetic construct
YTAIAWVKAFIRKLRK

SEQ ID NO: 46 - protein, 84 aa, synthetic construct
ARMEEMGSRTRDRLDEVKEAVAEVRAKLEEQAQQIRLQAEAFQARLKSWFEPLVEDMQRQWAGLVEKVQAAVGTSAAPVPSDNH

SEQ ID NO: 47 - protein, 84 aa, synthetic construct
ARMEEMGSRTRDRLDEVKEQVAEVRAKLEEQAQQIRLQAAAFQARLKSWFEPLVEDMQRQWAGLVEKVQAAVGTSAAPVPSDNH

SEQ ID NO: 48 - protein, 84 aa, synthetic construct
ARMEEMGSRTRDRLDEVKEQVAEVRAKLEEQAQQIRLQAEAFQARLKSWFEPLVEDMQRAWAGLVEKVQAAVGTSAAPVPSDNH

SEQ ID NO: 49 - protein, 84 aa, synthetic construct
ARMEEMGSRTRDRLDEVKEQVAEVRAKLEEQAQQIRLQAEAFQARLKSWFEPLVEDMQRQWAGLAEKVQAAVGTSAAPVPSDNH

SEQ ID NO: 50 - protein, 84 aa, synthetic construct
ARMEEMGSRTRDRLDEVKEQVAEVRAKLEEQAQQIRLQAEAFQARLKSWFEPLVEDMQRQWAGLVEKVQAAAGTSAAPVPSDNH

SEQ ID NO: 51 - protein, 84 aa, synthetic construct
ARMEEMGSRTRDRLDEVKEQVAEVRAKLEEQAQQIRLQAEAFQARLKSWFEPLVEDMQRQWAGLVEKVQAAVGTSAAPVASDNH

SEQ ID NO: 52 - protein, 84 aa, synthetic construct
ARMEEMGSRTRDRLDEVKEQVAEVRAKLEEQAQQIALQAEAFQARLKSWFEPLVEDMQRQWAGLVEKVQAAVGASAAPVPSDNH

SEQ ID NO: 53 - protein, 84 aa, synthetic construct
ARMEEMGSRARDRLAEVKEAVAEVAAKLEAQAQQARLQAAAFQAALKSWAEPLVADMQRAWAGLAEKVQAAVGTAAAPVASDNH

SEQ ID NO: 54 - protein, 84 aa, synthetic construct
ARMEEMGSRARDRLDEVKEAVAEVRAKLEAQAQQIRLQAAAFQARLKSWAEPLVEDMQRAWAGLVEKVQAAVGTSAAPVASDNH

SEQ ID NO: 55 - protein, 84 aa, synthetic construct
ARMEEMGSRTRDRLDEVKEAVAEVRAKLEEQAQQIRLQAAAFQARLKSWFEPLVEDMQRAWAGLVEKVQAAVGTSAAPVASDNH

SEQ ID NO: 56 - protein, 84 aa, synthetic construct
AAAAAMGSRTRDRLDEVKEQVAEVRAKLEEQAQQIRLQAEAFQARLKSWFEPLVEDMQRQWAGLVEKVQAAVGTSAAPVPSDNH

SEQ ID NO: 57 - protein, 84 aa, synthetic construct
ARMEEMGSRTRDRLDEVKEQVAEVRAKLEEQAQQIRLQAEAFQARLKSWFEPLVEDMQRQWAGLVEKVQAAVGTAAAAAAAAAA

SEQ ID NO: 58 - protein, 84 aa, synthetic construct
ARMEEMGSRTAAAAAEVKEQVAEVRAKLEEQAQQIRLQAEAFQARLKSWFEPLVEDMQRQWAGLVEKVQAAVGTSAAPVPSDNH

SEQ ID NO: 59 - protein, 84 aa, synthetic construct
ARMEEMGSRTRDRLDEVKEQVAAAAAALEEQAQQIRLQAEAFQARLKSWFEPLVEDMQRQWAGLVEKVQAAVGTSAAPVPSDNH

SEQ ID NO: 60 - protein, 331 aa, synthetic construct
KVEQAVETEPEPELRQQTEWQSGQRWELALGRFWDYLRWVQTLSEQVQEELLSSQVTQELRALMDETMKELKAYKSELEEQLTPVAEETRARLSKELQAAQARLGADMEDVCGRLVQYRGEVQAMLGQSTEELRVRLASHLRKLRKRLLRDADDLQKCLAVYQAGAREGAERGLSAIRERLGPLVEQGRVRAATVGSLAGQPLQERAQAWGERLRGSGGSDYKDHDGDYKDHDIDYKDDDDKSGSGSARMEEMGSRTRDRLDEVKEQVAEVRAKLEEQAQQIRLQAEAFQARLKSWFEPLVEDMQRQWAGLVEKVQAAVGTSAAPVPSDNH

SEQ ID NO: 61 - protein, 288 aa, synthetic construct
KVEQAVETEPEPELRQQTEWQSGQRWELALGRFWDYLRWVQTLSEQVQEELLSSQVTQELRALMDETMKELKAYKSELEEQLTPVAEETRARLSKELQAAQARLGADMEDVCGRLVQYRGEVQAMLGQSTEELRVRLASHLRKLRKRLLRDADDLQKCLAVYQAGAREGAERGLSAIRERLGPLVEQGRVRAATVGSLAGQPLQERAQAWGERLRARMEEMGSRTRDRLDEVKEQVAEVRAKLEAFQARLKSWFEPLVEDMQRQWAGLVEKVQAAVGTSAAPVPSDNH

SEQ ID NO: 62 - protein, 84 aa, synthetic construct
ARMEEMGSRTRDRLDEVKEQVAEVRAKLEEQAQQISLQAEAFQARLKSWFEPLVEDMQRQWAGLVEKVQAAVGASTAPVPSDNH

SEQ ID NO: 63 - protein, 9 aa, synthetic construct
RRRRRRRRR

SEQ ID NO: 64 - protein, 12 aa, synthetic construct
AAVLLPVLLAAP

SEQ ID NO: 65 - protein, 39 aa, synthetic construct
KSVRTWNEIIPSKGCLRVGGRCHPHVNGGGRRRRRRRRR

SEQ ID NO: 66 - protein, 18 aa, synthetic construct
MKVLWAALLVTFLAGCQA

SEQ ID NO: 67 - protein, 18 aa, synthetic construct
MKAAVLTLAVLFLTGSQA

SEQ ID NO: 68 - protein, 22 aa, synthetic construct
MMKTLLLFVGLLLTWESGQVLG

SEQ ID NO: 69 - protein, 4 aa, synthetic construct
SGGS

SEQ ID NO: 70 - protein, 5 aa, synthetic construct
GSSGS

SEQ ID NO: 71 - protein, 4 aa, synthetic construct
GGGS

SEQ ID NO: 72 - protein, 5 aa, synthetic construct
GGGGS

SEQ ID NO: 73 - protein, 5 aa, synthetic construct
SSSSG

SEQ ID NO: 74 - protein, 5 aa, synthetic construct
GSGSA

SEQ ID NO: 75 - protein, 5 aa, synthetic construct
GGSGG

SEQ ID NO: 76 - protein, 73 aa, synthetic construct
ARMEEMGSRTRDRLDEVKEQVAEVRAKLEAFQARLKSWFEPLVEDMQRQWAGLVEKVQAAVGTSAAPVPSDNH

SEQ ID NO: 77 - protein, 32 aa, synthetic construct
GSGGSDYKDHDGDYKDHDIDYKDDDDKSGSGS

SEQ ID NO: 78 - protein, 54 aa, synthetic construct
MGSRTRDRLDEVKEQVAEVRAKLEEQAQQIRLQAEAFQARLKSWFEPLVEDMQR

SEQ ID NO: 79 - protein, 167 aa, synthetic construct
KVEQAVETEPEPELRQQTEWQSGQRWELALGRFWDYLRWVQTLSEQVQEELLSSQVTQELRALMDETMKELKAYKSELEEQLTPVAEETRARLSKELQAAQARLGADMEDVCGRLVQYRGEVQAMLGQSTEELRVRLASHLRKLRKRLLRDADDLQKCLAVYQAGAR

SEQ ID NO: 80 - protein, 38 aa, synthetic construct
EGAERGLSAIRERLGPLVEQGRVRAATVGSLAGQPLQE

SEQ ID NO: 81 - protein, 205 aa, synthetic construct
KVEQAVETEPEPELRQQTEWQSGQRWELALGRFWDYLRWVQTLSEQVQEELLSSQVTQELRALMDETMKELKAYKSELEEQLTPVAEETRARLSKELQAAQARLGADMEDVCGRLVQYRGEVQAMLGQSTEELRVRLASHLRKLRKRLLRDADDLQKCLAVYQAGAREGAERGLSAIRERLGPLVEQGRVRAATVGSLAGQPLQE

SEQ ID NO: 82 - protein, 14 aa, synthetic construct
GKPIPNPLLGLDST

SEQ ID NO: 83 - protein, 9 aa, synthetic construct
IPNPLLGLD

SEQ ID NO: 84 - protein, 10 aa, synthetic construct
RRRRRRRRRR

SEQ ID NO: 85 - protein, 11 aa, synthetic construct
RRRRRRRRRRR

SEQ ID NO: 86 - protein, 12 aa, synthetic construct
RRRRRRRRRRRR

SEQ ID NO: 87 - protein, 55 aa, synthetic construct
EMGSRTRDRLDEVKEQVAEVRAKLEEQAQQIRLQAEAFQARLKSWFEPLVEDMQR

SEQ ID NO: 88 - protein, 8 aa, synthetic construct
GGGSGGGS

SEQ ID NO: 89 - protein, 299 aa, Homo sapiens
KVEQAVETEPEPELRQQTEWQSGQRWELALGRFWDYLRWVQTLSEQVQEELLSSQVTQELRALMDETMKELKAYKSELEEQLTPVAEETRARLSKELQAAQARLGADMEDVCGRLVQYRGEVQAMLGQSTEELRVRLASHLRKLRKRLLRDADDLQKRLAVYQAGAREGAERGLSAIRERLGPLVEQGRVRAATVGSLAGQPLQERAQAWGERLRARMEEMGSRTRDRLDEVKEQVAEVRAKLEEQAQQIRLQAEAFQARLKSWFEPLVEDMQRQWAGLVEKVQAAVGTSAAPVPSDNH

SEQ ID NO: 90 - protein, 167 aa, synthetic construct
KVEQAVETEPEPELRQQTEWQSGQRWELALGRFWDYLRWVQTLSEQVQEELLSSQVTQELRALMDETMKELKAYKSELEEQLTPVAEETRARLSKELQAAQARLGADMEDVCGRLVQYRGEVQAMLGQSTEELRVRLASHLRKLRKRLLRDADDLQKRLAVYQAGAR

SEQ ID NO: 91 - DNA, 20 bp, synthetic construct
  source 1..20: mol_type = other DNA
attatctaatggacgacccc

SEQ ID NO: 92 - DNA, 20 bp, synthetic construct
  source 1..20: mol_type = other DNA
caaatacggagcgaagcacg

SEQ ID NO: 93 - DNA, 21 bp, synthetic construct
  source 1..21: mol_type = other DNA
agagcaacatctggggacaaa

SEQ ID NO: 94 - DNA, 22 bp, synthetic construct
  source 1..22: mol_type = other DNA
tccacaaataggttggccagat

SEQ ID NO: 95 - DNA, 20 bp, synthetic construct
  source 1..20: mol_type = other DNA
aacgaattggctttgctgtc

SEQ ID NO: 96 - DNA, 21 bp, synthetic construct
  source 1..21: mol_type = other DNA
aggctatggtcatgagggttg

SEQ ID NO: 97 - DNA, 20 bp, synthetic construct
  source 1..20: mol_type = other DNA
tgactctctgcatggtggtg

SEQ ID NO: 98 - DNA, 20 bp, synthetic construct
  source 1..20: mol_type = other DNA
tcagaattgagtgcagggct

SEQ ID NO: 99 - DNA, 20 bp, synthetic construct
  source 1..20: mol_type = other DNA
tttgagcctcccttgactgg

SEQ ID NO: 100 - DNA, 19 bp, synthetic construct
  source 1..19: mol_type = other DNA
ggtattccagtccccgctg